European Patent Specification EP 3 233 915 B1, published August 28, 2024. Title: Antibodies for IL-17C. Applicant: MorphoSys AG Galapagos NV. The sequence listing filed with the application follows.

SEQUENCE LISTING (31 sequences)

SEQ ID NO: 1 - protein, 197 aa, Homo sapiens
MTLLPGLLFLTWLHTCLAHHDPSLRGHPHSHGTPHCYSAEELPLGQAPPHLLARGAKWGQALPVALVSSLEAASHRGRHERPSATTQCPVLRPEEVLEADTHQRSISPWRYRVDTDEDRYPQKLAFAECLCRGCIDARTGRETAALNSVRLLQSLLVLRRRPCSRDGSGLPTPGAFAFHTEFIHVPVGCTCVLPRSV

SEQ ID NO: 2 - protein, 194 aa, Mus musculus
MSLLLLGWLPTGMTHQDPPSWGKPRSHRTLRCYSAEELSHGQAPPHLLTRSARWEQALPVALVASLEATGHRRQHEGPLAGTQCPVLRPEEVLEADTHERSISPWRYRIDTDENRYPQKLAVAECLCRGCINAKTGRETAALNSVQLLQSLLVLRRQPCSRDGTADPTPGSFAFHTEFIRVPVGCTCVLPRSTQ

SEQ ID NO: 3 - protein, 197 aa, Macaca fascicularis
MTLLPGLLFLTWLHACLAHQDPFLRGHPHTHGTPRCYSAEELPLGQAPPHLLARGAKWGQALPVALVSSLEAAGHRRRHDRPSAATQCPVLRPEEVLEADTHQRSISPWRYRVDTDEDRYPQKLAFAECLCRGCIDPRTGRETAALNSVRLLQSLLVLRRRPCSRDGSGLPTPGAFAFHTEFIRVPVGCTCVLPRSV

SEQ ID NO: 4 - protein, 866 aa, Homo sapiens
MGAARSPPSAVPGPLLGLLLLLLGVLAPGGASLRLLDHRALVCSQPGLNCTVKNSTCLDDSWIHPRNLTPSSPKDLQIQLHFAHTQQGDLFPVAHIEWTLQTDASILYLEGAELSVLQLNTNERLCVRFEFLSKLRHHHRRWRFTFSHFVVDPDQEYEVTVHHLPKPIPDGDPNHQSKNFLVPDCEHARMKVTTPCMSSGSLWDPNITVETLEAHQLRVSFTLWNESTHYQILLTSFPHMENHSCFEHMHHIPAPRPEEFHQRSNVTLTLRNLKGCCRHQVQIQPFFSSCLNDCLRHSATVSCPEMPDTPEPIPDYMPLWVYWFITGISILLVGSVILLIVCMTWRLAGPGSEKYSDDTKYTDGLPAADLIPPPLKPRKVWIIYSADHPLYVDVVLKFAQFLLTACGTEVALDLLEEQAISEAGVMTWVGRQKQEMVESNSKIIVLCSRGTRAKWQALLGRGAPVRLRCDHGKPVGDLFTAAMNMILPDFKRPACFGTYVVCYFSEVSCDGDVPDLFGAAPRYPLMDRFEEVYFRIQDLEMFQPGRMHRVGELSGDNYLRSPGGRQLRAALDRFRDWQVRCPDWFECENLYSADDQDAPSLDEEVFEEPLLPPGTGIVKRAPLVREPGSQACLAIDPLVGEEGGAAVAKLEPHLQPRGQPAPQPLHTLVLAAEEGALVAAVEPGPLADGAAVRLALAGEGEACPLLGSPGAGRNSVLFLPVDPEDSPLGSSTPMASPDLLPEDVREHLEGLMLSLFEQSLSCQAQGGCSRPAMVLTDPHTPYEEEQRQSVQSDQGYISRSSPQPPEGLTEMEEEEEEEQDPGKPALPLSPEDLESLRSLQRQLLFRQLQKNSGWDTMGSESEGPSA

SEQ ID NO: 5 - protein, 667 aa, Homo sapiens
MGSSRLAALLLPLLLIVIDLSDSAGIGFRHLPHWNTRCPLASHTDDSFTGSSAYIPCRTWWALFSTKPWCVRVWHCSRCLCQHLLSGGSGLQRGLFHLLVQKSKKSSTFKFYRRHKMPAPAQRKLLPRRHLSEKSHHISIPSPDISHKGLRSKRTQPSDPETWESLPRLDSQRHGGPEFSFDLLPEARAIRVTISSGPEVSVRLCHQWALECEELSSPYDVQKIVSGGHTVELPYEFLLPCLCIEASYLQEDTVRRKKCPFQSWPEAYGSDFWKSVHFTDYSQHTQMVMALTLRCPLKLEAALCQRHDWHTLCKDLPNATARESDGWYVLEKVDLHPQLCFKFSFGNSSHVECPHQTGSLTSWNVSMDTQAQQLILHFSSRMHATFSAAWSLPGLGQDTLVPPVYTVSQARGSSPVSLDLIIPFLRPGCCVLVWRSDVQFAWKHLLCPDVSYRHLGLLILALLALLTLLGVVLALTCRRPQSGPGPARPVLLLHAADSEAQRRLVGALAELLRAALGGGRDVIVDLWEGRHVARVGPLPWLWAARTRVAREQGTVLLLWSGADLRPVSGPDPRAAPLLALLHAAPRPLLLLAYFSRLCAKGDIPPPLRALPRYRLLRDLPRLLRALDARPFAEATSWGRLGARQRRQSRLELCSRLEREAARLADLG

SEQ ID NO: 6 - protein, 637 aa, Mus musculus
MGSPRLAALLLSLPLLLIGLAVSARVACPCLRSWTSHCLLAYRVDKRFAGLQWGWFPLLVRKSKSPPKFEDYWRHRTPASFQRKLLGSPSLSEESHRISIPSSAISHRGQRTKRAQPSAAEGREHLPEAGSQKCGGPEFSFDLLPEVQAVRVTIPAGPKASVRLCYQWALECEDLSSPFDTQKIVSGGHTVDLPYEFLLPCMCIEASYLQEDTVRRKKCPFQSWPEAYGSDFWQSIRFTDYSQHNQMVMALTLRCPLKLEASLCWRQDPLTPCETLPNATAQESEGWYILENVDLHPQLCFKFSFENSSHVECPHQSGSLPSWTVSMDTQAQQLTLHFSSRTYATFSAAWSDPGLGPDTPMPPVYSISQTQGSVPVTLDLIIPFLRQENCILVWRSDVHFAWKHVLCPDVSHRHLGLLILALLALTALVGVVLVLLGRRLLPGSGRTRPVLLLHAADSEAQRRLVGALAELLRTALGGGRDVIVDLWEGTHVARIGPLPWLWAARERVAREQGTVLLLWNCAGPSTACSGDPQAASLRTLLCAAPRPLLLAYFSRLCAKGDIPRPLRALPRYRLLRDLPRLLRALDAQPATLASSWSHLGAKRCLKNRLEQCHLLELEAAKDDYQGSTNSPCGFSCL

SEQ ID NO: 7 - protein, 9 aa, Artificial Sequence
  derived from recombinant library
FTFSSYAMS

SEQ ID NO: 8 - protein, 19 aa, Artificial Sequence
  derived from recombinant library
VSAISGSGGSTYYADSVKG

SEQ ID NO: 9 - protein, 11 aa, Artificial Sequence
  derived from recombinant library
GFRGGFFAFDV

SEQ ID NO: 10 - protein, 11 aa, Artificial Sequence
  derived from recombinant library
SGDKLGDKYAY

SEQ ID NO: 11 - protein, 11 aa, Artificial Sequence
  derived from recombinant library
LVIYQDSKRPS

SEQ ID NO: 12 - protein, 10 aa, Artificial Sequence
  derived from recombinant library
QAWTFPLLTW

SEQ ID NO: 13 - protein, 214 aa, Artificial Sequence
  derived from recombinant library
SYELTQPPSVSVSPGQTASITCSGDKLGDKYAYWYQQKPGQSPVLVIYQDSKRPSGIPERFSGSNSGNTATLTISGTQAEDEADYYCQAWTFPLLTWVFGGGTKLTVLGQPKAAPSVTLFPPSSEELQANKATLVCLISDFYPGAVTVAWKADSSPVKAGVETTTPSKQSNNKYAASSYLSLTPEQWKSHRSYSCQVTHEGSTVEKTVAPTECS

SEQ ID NO: 14 - protein, 450 aa, Artificial Sequence
  derived from recombinant library
EVQLLESGGGLVQPGGSLRLSCAASGFTFSSYAMSWVRQAPGKGLEWVSAISGSGGSTYYADSVKGRFTISRDNSKNTLYLQMNSLRAEDTAVYYCARGFRGGFFAFDVWGQGTLVTVSSASTKGPSVFPLAPSSKSTSGGTAALGCLVKDYFPEPVTVSWNSGALTSGVHTFPAVLQSSGLYSLSSVVTVPSSSLGTQTYICNVNHKPSNTKVDKRVEPKSCDKTHTCPPCPAPELLGGPSVFLFPPKPKDTLMISRTPEVTCVVVDVSHEDPEVKFNWYVDGVEVHNAKTKPREEQYNSTYRVVSVLTVLHQDWLNGKEYKCKVSNKALPAPIEKTISKAKGQPREPQVYTLPPSREEMTKNQVSLTCLVKGFYPSDIAVEWESNGQPENNYKTTPPVLDSDGSFFLYSKLTVDKSRWQQGNVFSCSVMHEALHNHYTQKSLSLSPGK

SEQ ID NO: 15 - DNA, 642 bp, Artificial Sequence
  derived from recombinant library
agctatgaactgacccagccgccgagcgttagcgttagcccaggccagaccgccagcattacctgtagcggcgacaaactgggcgacaaatacgcctactggtatcagcagaaaccgggccagagcccggtgctggttatctatcaggatagcaaacgcccgagcggcattccagaacgctttagcggcagcaacagcggcaacaccgccaccctgaccattagcggcacccaggccgaagacgaagccgattattactgccaggcttggactttcccgctgctgacttgggtgtttggcggcggtaccaagctgaccgtgctgggccagcccaaagccgcccctagcgtgaccctgttccccccaagcagcgaggaactccaggccaacaaggccaccctcgtgtgcctgatcagcgacttctaccctggcgccgtgaccgtggcctggaaggccgatagcagccctgtgaaggccggcgtggaaaccaccacccccagcaagcagagcaacaacaaatacgccgccagcagctacctgagcctgacccccgagcagtggaagtcccacagatcctacagctgccaggtcacacacgagggcagcaccgtggaaaagaccgtggcccccaccgagtgcagc

SEQ ID NO: 16 - DNA, 1350 bp, Artificial Sequence
  derived from recombinant library
gaagtgcagctgctggaaagcggtggcggtctggtgcagccaggtggtagcctgcgcctgagctgtgccgcaagcggctttacctttagcagctatgccatgagctgggtgcgccaagcaccaggcaaaggcctggaatgggtgagcgccattagcggcagcggtggcagcacctattatgccgatagcgtgaaaggtcgctttaccattagtcgcgataacagcaaaaacaccctgtatctgcaaatgaacagcctgcgggcagaagataccgcagtttattattgcgcgcgaggattccgtggtggtttcttcgcattcgatgtgtggggtcagggcaccctggttactgtctcgagcgcgtcgaccaaaggccccagcgtgttccctctggcccccagcagcaagagcacctctggcggaacagccgccctgggctgcctggtcaaggactacttccccgagcccgtgaccgtgtcctggaactctggcgccctgaccagcggcgtgcacacctttccagccgtgctccagagcagcggcctgtacagcctgagcagcgtcgtgaccgtgcccagcagcagcctgggcacccagacctacatctgcaacgtgaaccacaagcccagcaacacaaaggtggacaagcgggtggaacccaagagctgcgacaagacccacacctgtcccccctgccctgcccctgaactgctgggaggcccctccgtgttcctgttccccccaaagcctaaggacaccctgatgatcagccggacccccgaagtgacctgcgtggtggtggacgtgtcccacgaggaccctgaagtgaagtttaattggtacgtggacggcgtggaagtgcacaacgccaagaccaagcccagagaggaacagtacaacagcacctaccgggtggtgtccgtgctgaccgtgctgcaccaggactggctgaacggcaaagagtacaagtgcaaggtgtccaacaaggccctgcctgcccccatcgagaaaaccatcagcaaggccaaaggccagccccgcgagccccaggtgtacacactgccccctagccgggaagagatgaccaagaaccaggtgtccctgacctgcctcgtgaagggcttctaccccagcgacattgccgtggaatgggagagcaacggccagcccgagaacaactacaagaccaccccccctgtgctggacagcgacggctcattcttcctgtacagcaagctgaccgtggacaagagccggtggcagcagggcaacgtgttcagctgctccgtgatgcacgaggccctgcacaaccactacacccagaagtccctgagcctgagccccggcaag

SEQ ID NO: 17 - protein, 9 aa, Artificial Sequence
  derived from recombinant library
FTFSSYAMS

SEQ ID NO: 18 - protein, 19 aa, Artificial Sequence
  derived from recombinant library
VSAISGSGGSTYYADSVKG

SEQ ID NO: 19 - protein, 11 aa, Artificial Sequence
  derived from recombinant library
GFAIRYYGFDY

SEQ ID NO: 20 - protein, 11 aa, Artificial Sequence
  derived from recombinant library
SGDKLGDKYAY

SEQ ID NO: 21 - protein, 11 aa, Artificial Sequence
  derived from recombinant library
LVIYQDSKRPS

SEQ ID NO: 22 - protein, 10 aa, Artificial Sequence
  derived from recombinant library
QVFTFPLVTT

SEQ ID NO: 23 - protein, 214 aa, Artificial Sequence
  derived from recombinant library
SYELTQPPSVSVSPGQTASITCSGDKLGDKYAYWYQQKPGQSPVLVIYQDSKRPSGIPERFSGSNSGNTATLTISGTQAEDEADYYCQVFTFPLVTTVFGGGTKLTVLGQPKAAPSVTLFPPSSEELQANKATLVCLISDFYPGAVTVAWKADSSPVKAGVETTTPSKQSNNKYAASSYLSLTPEQWKSHRSYSCQVTHEGSTVEKTVAPTECS

SEQ ID NO: 24 - protein, 450 aa, Artificial Sequence
  derived from recombinant library
EVQLLESGGGLVQPGGSLRLSCAASGFTFSSYAMSWVRQAPGKGLEWVSAISGSGGSTYYADSVKGRFTISRDNSKNTLYLQMNSLRAEDTAVYYCARGFAIRYYGFDYWGQGTLVTVSSASTKGPSVFPLAPSSKSTSGGTAALGCLVKDYFPEPVTVSWNSGALTSGVHTFPAVLQSSGLYSLSSVVTVPSSSLGTQTYICNVNHKPSNTKVDKRVEPKSCDKTHTCPPCPAPELLGGPSVFLFPPKPKDTLMISRTPEVTCVVVDVSHEDPEVKFNWYVDGVEVHNAKTKPREEQYNSTYRVVSVLTVLHQDWLNGKEYKCKVSNKALPAPIEKTISKAKGQPREPQVYTLPPSREEMTKNQVSLTCLVKGFYPSDIAVEWESNGQPENNYKTTPPVLDSDGSFFLYSKLTVDKSRWQQGNVFSCSVMHEALHNHYTQKSLSLSPGK

SEQ ID NO: 25 - DNA, 642 bp, Artificial Sequence
  derived from recombinant library
agctatgaactgacccagccgccgagcgttagcgttagcccaggccagaccgccagcattacctgtagcggcgacaaactgggcgacaaatacgcctactggtatcagcagaaaccgggccagagcccggtgctggttatctatcaggatagcaaacgcccgagcggcattccagaacgctttagcggcagcaacagcggcaacaccgccaccctgaccattagcggcacccaggccgaagacgaagccgattattactgccaggttttcactttcccgctggttactactgtgtttggcggcggtaccaagctgaccgtgctgggccagcccaaagccgcccctagcgtgaccctgttccccccaagcagcgaggaactccaggccaacaaggccaccctcgtgtgcctgatcagcgacttctaccctggcgccgtgaccgtggcctggaaggccgatagcagccctgtgaaggccggcgtggaaaccaccacccccagcaagcagagcaacaacaaatacgccgccagcagctacctgagcctgacccccgagcagtggaagtcccacagatcctacagctgccaggtcacacacgagggcagcaccgtggaaaagaccgtggcccccaccgagtgcagc

SEQ ID NO: 26 - DNA, 1350 bp, Artificial Sequence
  derived from recombinant library
gaagtgcagctgctggaaagcggtggcggtctggtgcagccaggtggtagcctgcgcctgagctgtgccgcaagcggctttacctttagcagctatgccatgagctgggtgcgccaagcaccaggcaaaggcctggaatgggtgagcgccattagcggcagcggtggcagcacctattatgccgatagcgtgaaaggtcgctttaccattagtcgcgataacagcaaaaacaccctgtatctgcaaatgaacagcctgcgggcagaagataccgcagtttattattgcgcgcgtggtttcgcaatccgttattatggatttgattattggggccagggcaccctggttactgtctcgagcgcgtcgaccaaaggccccagcgtgttccctctggcccccagcagcaagagcacctctggcggaacagccgccctgggctgcctggtcaaggactacttccccgagcccgtgaccgtgtcctggaactctggcgccctgaccagcggcgtgcacacctttccagccgtgctccagagcagcggcctgtacagcctgagcagcgtcgtgaccgtgcccagcagcagcctgggcacccagacctacatctgcaacgtgaaccacaagcccagcaacacaaaggtggacaagcgggtggaacccaagagctgcgacaagacccacacctgtcccccctgccctgcccctgaactgctgggaggcccctccgtgttcctgttccccccaaagcctaaggacaccctgatgatcagccggacccccgaagtgacctgcgtggtggtggacgtgtcccacgaggaccctgaagtgaagtttaattggtacgtggacggcgtggaagtgcacaacgccaagaccaagcccagagaggaacagtacaacagcacctaccgggtggtgtccgtgctgaccgtgctgcaccaggactggctgaacggcaaagagtacaagtgcaaggtgtccaacaaggccctgcctgcccccatcgagaaaaccatcagcaaggccaaaggccagccccgcgagccccaggtgtacacactgccccctagccgggaagagatgaccaagaaccaggtgtccctgacctgcctcgtgaagggcttctaccccagcgacattgccgtggaatgggagagcaacggccagcccgagaacaactacaagaccaccccccctgtgctggacagcgacggctcattcttcctgtacagcaagctgaccgtggacaagagccggtggcagcagggcaacgtgttcagctgctccgtgatgcacgaggccctgcacaaccactacacccagaagtccctgagcctgagccccggcaag

SEQ ID NO: 27 - protein, 9 aa, Homo sapiens
PVLRPEEVL

SEQ ID NO: 28 - protein, 8 aa, Homo sapiens
VLRPEEVL

SEQ ID NO: 29 - protein, 13 aa, Homo sapiens
ADTHQRSISPWRY

SEQ ID NO: 30 - protein, 16 aa, Homo sapiens
CRGCIDARTGRETAAL

SEQ ID NO: 31 - protein, 8 aa, Homo sapiens
TCVLPRSV